European Patent Application EP 4 286 393 A1, published December 6, 2023. Title: New Method for Producing Antibody-Immunostimulant Conjugate. Applicant: DAIICHI SANKYO COMPANY, LIMITED. The sequence listing filed with the application follows.

SEQUENCE LISTING (68 sequences)

SEQ ID NO: 1 - protein, 218 aa, Artificial Sequence
  Anti-CD70 Antibody 1 Light Chain
DIVMTQSPDSLAVSLGERATINCRASKSVSTSGYSFMHWYQQKPGQPPKLLIYLASNLESGVPDRFSGSGSGTDFTLTISSLQAEDVAVYYCQHSREVPWTFGQGTKVEIKRTVAAPSVFIFPPSDEQLKSGTASVVCLLNNFYPREAKVQWKVDNALQSGNSQESVTEQDSKDSTYSLSSTLTLSKADYEKHKVYACEVTHQGLSSPVTKSFNRGEC

SEQ ID NO: 2 - protein, 448 aa, Artificial Sequence
  Anti-CD70 Antibody 1 Heavy Chain
QVQLVQSGAEVKKPGASVKVSCKASGYTFTNYGMNWVRQAPGQGLKWMGWINTYTGEPTYADAFKGRVTMTRDTSISTAYMELSRLRSDDTAVYYCARDYGDYGMDYWGQGTTVTVSSASTKGPSVFPLAPSSKSTSGGTAALGCLVKDYFPEPVTVSWNSGALTSGVHTFPAVLQSSGLYSLSSVVTVPSSSLGTQTYICNVNHKPSNTKVDKRVEPKSCDKTHTCPPCPAPEAAGGPSVFLFPPKPKDTLMISRTPEVTCVVVDVSHEDPEVKFNWYVDGVEVHNAKTKPREEQYNSTYRVVSVLTVLHQDWLNGKEYKCKVSNKALPAPIEKTISKAKGQPREPQVYTLPPSREEMTKNQVSLTCLVKGFYPSDIAVEWESNGQPENNYKTTPPVLDSDGSFFLYSKLTVDKSRWQQGNVFSCSVMHEALHNHYTQKSLSLSPGK

SEQ ID NO: 3 - protein, 214 aa, Artificial Sequence
  Anti-CD70 Antibody 2 Light Chain
EIVLTQSPATLSLSPGERATLSCRASQSVSSYLAWYQQKPGQAPRLLIYDASNRATGIPARFSGSGSGTDFTLTISSLEPEDFAVYYCQQRTNWPLTFGGGTKVEIKRTVAAPSVFIFPPSDEQLKSGTASVVCLLNNFYPREAKVQWKVDNALQSGNSQESVTEQDSKDSTYSLSSTLTLSKADYEKHKVYACEVTHQGLSSPVTKSFNRGEC

SEQ ID NO: 4 - protein, 448 aa, Artificial Sequence
  Anti-CD70 Antibody 2 Heavy Chain
QVQLVESGGGVVQPGRSLRLSCAASGFTFSSYIMHWVRQAPGKGLEWVAVISYDGRNKYYADSVKGRFTISRDNSKNTLYLQMNSLRAEDTAVYYCARDTDGYDFDYWGQGTLVTVSSASTKGPSVFPLAPSSKSTSGGTAALGCLVKDYFPEPVTVSWNSGALTSGVHTFPAVLQSSGLYSLSSVVTVPSSSLGTQTYICNVNHKPSNTKVDKRVEPKSCDKTHTCPPCPAPEAAGGPSVFLFPPKPKDTLMISRTPEVTCVVVDVSHEDPEVKFNWYVDGVEVHNAKTKPREEQYNSTYRVVSVLTVLHQDWLNGKEYKCKVSNKALPAPIEKTISKAKGQPREPQVYTLPPSREEMTKNQVSLTCLVKGFYPSDIAVEWESNGQPENNYKTTPPVLDSDGSFFLYSKLTVDKSRWQQGNVFSCSVMHEALHNHYTQKSLSLSPGK

SEQ ID NO: 5 - protein, 214 aa, Artificial Sequence
  Anti-TROP2 Antibody 1 Light Chain
DIQMTQSPSSLSASVGDRVTITCKASQDVSTAVAWYQQKPGKAPKLLIYSASYRYTGVPSRFSGSGSGTDFTLTISSLQPEDFAVYYCQQHYITPLTFGQGTKLEIKRTVAAPSVFIFPPSDEQLKSGTASVVCLLNNFYPREAKVQWKVDNALQSGNSQESVTEQDSKDSTYSLSSTLTLSKADYEKHKVYACEVTHQGLSSPVTKSFNRGEC

SEQ ID NO: 6 - protein, 451 aa, Artificial Sequence
  Anti-TROP2 Antibody 1 Heavy Chain
QVQLVQSGAEVKKPGASVKVSCKASGYTFTTAGMQWVRQAPGQGLEWMGWINTHSGVPKYAEDFKGRVTISADTSTSTAYLQLSSLKSEDTAVYYCARSGFGSSYWYFDVWGQGTLVTVSSASTKGPSVFPLAPSSKSTSGGTAALGCLVKDYFPEPVTVSWNSGALTSGVHTFPAVLQSSGLYSLSSVVTVPSSSLGTQTYICNVNHKPSNTKVDKRVEPKSCDKTHTCPPCPAPELLGGPSVFLFPPKPKDTLMISRTPEVTCVVVDVSHEDPEVKFNWYVDGVEVHNAKTKPREEQYNSTYRVVSVLTVLHQDWLNGKEYKCKVSNKALPAPIEKTISKAKGQPREPQVYTLPPSREEMTKNQVSLTCLVKGFYPSDIAVEWESNGQPENNYKTTPPVLDSDGSFFLYSKLTVDKSRWQQGNVFSCSVMHEALHNHYTQKSLSLSPGK

SEQ ID NO: 7 - protein, 214 aa, Artificial Sequence; identical to SEQ ID NO: 5
  Anti-TROP2 Antibody 2 Light Chain

SEQ ID NO: 8 - protein, 451 aa, Artificial Sequence
  Anti-TROP2 Antibody 2 Heavy Chain
QVQLVQSGAEVKKPGASVKVSCKASGYTFTTAGMQWVRQAPGQGLEWMGWINTHSGVPKYAEDFKGRVTISADTSTSTAYLQLSSLKSEDTAVYYCARSGFGSSYWYFDVWGQGTLVTVSSASTKGPSVFPLAPSSKSTSGGTAALGCLVKDYFPEPVTVSWNSGALTSGVHTFPAVLQSSGLYSLSSVVTVPSSSLGTQTYICNVNHKPSNTKVDKRVEPKSCDKTHTCPPCPAPEAAGGPSVFLFPPKPKDTLMISRTPEVTCVVVDVSHEDPEVKFNWYVDGVEVHNAKTKPREEQYNSTYRVVSVLTVLHQDWLNGKEYKCKVSNKALPAPIEKTISKAKGQPREPQVYTLPPSREEMTKNQVSLTCLVKGFYPSDIAVEWESNGQPENNYKTTPPVLDSDGSFFLYSKLTVDKSRWQQGNVFSCSVMHEALHNHYTQKSLSLSPGK

SEQ ID NO: 9 - protein, 214 aa, Artificial Sequence
  Anti-EGFR Antibody 1 Light Chain
DIQMTQSPSSLSASVGDRVTITCQASQDISNYLNWYQQKPGKAPKLLIYDASNLETGVPSRFSGSGSGTDFTFTISSLQPEDIATYFCQHFDHLPLAFGGGTKVEIKRTVAAPSVFIFPPSDEQLKSGTASVVCLLNNFYPREAKVQWKVDNALQSGNSQESVTEQDSKDSTYSLSSTLTLSKADYEKHKVYACEVTHQGLSSPVTKSFNRGEC

SEQ ID NO: 10 - protein, 449 aa, Artificial Sequence
  Anti-EGFR Antibody 1 Heavy Chain
QVQLQESGPGLVKPSETLSLTCTVSGGSVSSGDYYWTWIRQSPGKGLEWIGHIYYSGNTNYNPSLKSRLTISIDTSKTQFSLKLSSVTAADTAIYYCVRDRVTGAFDIWGQGTMVTVSSASTKGPSVFPLAPSSKSTSGGTAALGCLVKDYFPEPVTVSWNSGALTSGVHTFPAVLQSSGLYSLSSVVTVPSSSLGTQTYICNVNHKPSNTKVDKRVEPKSCDKTHTCPPCPAPEAAGGPSVFLFPPKPKDTLMISRTPEVTCVVVDVSHEDPEVKFNWYVDGVEVHNAKTKPREEQYNSTYRVVSVLTVLHQDWLNGKEYKCKVSNKALPAPIEKTISKAKGQPREPQVYTLPPSREEMTKNQVSLTCLVKGFYPSDIAVEWESNGQPENNYKTTPPVLDSDGSFFLYSKLTVDKSRWQQGNVFSCSVMHEALHNHYTQKSLSLSPGK

SEQ ID NO: 11 - protein, 214 aa, Artificial Sequence
  Anti-EGFR Antibody 2 Light Chain
DILMTQSPSSMSVSLGDTVSITCHSSQDINSNIGWLQQRPGKSFKGLIYHGTNLDDEVPSRFSGSGSGADYSLTISSLESEDFADYYCVQYAQFPWTFGGGTKLEIKRTVAAPSVFIFPPSDEQLKSGTASVVCLLNNFYPREAKVQWKVDNALQSGNSQESVTEQDSKDSTYSLSSTLTLSKADYEKHKVYACEVTHQGLSSPVTKSFNRGEC

SEQ ID NO: 12 - protein, 446 aa, Artificial Sequence
  Anti-EGFR Antibody 2 Heavy Chain
DVQLQESGPSLVKPSQSLSLTCTVTGYSITSDFAWNWIRQFPGNKLEWMGYISYSGNTRYNPSLKSRISITRDTSKNQFFLQLNSVTIEDTATYYCVTAGRGFPYWGQGTLVTVSAASTKGPSVFPLAPSSKSTSGGTAALGCLVKDYFPEPVTVSWNSGALTSGVHTFPAVLQSSGLYSLSSVVTVPSSSLGTQTYICNVNHKPSNTKVDKRVEPKSCDKTHTCPPCPAPEAAGGPSVFLFPPKPKDTLMISRTPEVTCVVVDVSHEDPEVKFNWYVDGVEVHNAKTKPREEQYNSTYRVVSVLTVLHQDWLNGKEYKCKVSNKALPAPIEKTISKAKGQPREPQVYTLPPSREEMTKNQVSLTCLVKGFYPSDIAVEWESNGQPENNYKTTPPVLDSDGSFFLYSKLTVDKSRWQQGNVFSCSVMHEALHNHYTQKSLSLSPGK

SEQ ID NO: 13 - protein, 15 aa, Artificial Sequence
  Anti-CD70 Antibody 1 CDRL1
RASKSVSTSGYSFMH

SEQ ID NO: 14 - protein, 7 aa, Artificial Sequence
  Anti-CD70 Antibody 1 CDRL2
LASNLES

SEQ ID NO: 15 - protein, 9 aa, Artificial Sequence
  Anti-CD70 Antibody 1 CDRL3
QHSREVPWT

SEQ ID NO: 16 - protein, 10 aa, Artificial Sequence
  Anti-CD70 Antibody 1 CDRH1
GYTFTNYGMN

SEQ ID NO: 17 - protein, 17 aa, Artificial Sequence
  Anti-CD70 Antibody 1 CDRH2
WINTYTGEPTYADAFKG

SEQ ID NO: 18 - protein, 9 aa, Artificial Sequence
  Anti-CD70 Antibody 1 CDRH3
DYGDYGMDY

SEQ ID NO: 19 - protein, 11 aa, Artificial Sequence
  Anti-CD70 Antibody 2 CDRL1
RASQSVSSYLA

SEQ ID NO: 20 - protein, 7 aa, Artificial Sequence
  Anti-CD70 Antibody 2 CDRL2
DASNRAT

SEQ ID NO: 21 - protein, 9 aa, Artificial Sequence
  Anti-CD70 Antibody 2 CDRL3
QQRTNWPLT

SEQ ID NO: 22 - protein, 5 aa, Artificial Sequence
  Anti-CD70 Antibody 2 CDRH1
SYIMH

SEQ ID NO: 23 - protein, 17 aa, Artificial Sequence
  Anti-CD70 Antibody 2 CDRH2
VISYDGRNKYYADSVKG

SEQ ID NO: 24 - protein, 9 aa, Artificial Sequence
  Anti-CD70 Antibody 2 CDRH3
DTDGYDFDY

SEQ ID NO: 25 - protein, 11 aa, Artificial Sequence
  Anti-TROP2 Antibody 1 CDRL1
KASQDVSTAVA

SEQ ID NO: 26 - protein, 7 aa, Artificial Sequence
  Anti-TROP2 Antibody 1 CDRL2
SASYRYT

SEQ ID NO: 27 - protein, 9 aa, Artificial Sequence
  Anti-TROP2 Antibody 1 CDRL3
QQHYITPLT

SEQ ID NO: 28 - protein, 5 aa, Artificial Sequence
  Anti-TROP2 Antibody 1 CDRH1
TAGMQ

SEQ ID NO: 29 - protein, 17 aa, Artificial Sequence
  Anti-TROP2 Antibody 1 CDRH2
WINTHSGVPKYAEDFKG

SEQ ID NO: 30 - protein, 12 aa, Artificial Sequence
  Anti-TROP2 Antibody 1 CDRH3
SGFGSSYWYFDV

SEQ ID NO: 31 - protein, 11 aa, Artificial Sequence
  Anti-TROP2 Antibody 2 CDRL1
KASQDVSTAVA

SEQ ID NO: 32 - protein, 7 aa, Artificial Sequence
  Anti-TROP2 Antibody 2 CDRL2
SASYRYT

SEQ ID NO: 33 - protein, 9 aa, Artificial Sequence
  Anti-TROP2 Antibody 2 CDRL3
QQHYITPLT

SEQ ID NO: 34 - protein, 5 aa, Artificial Sequence
  Anti-TROP2 Antibody 2 CDRH1
TAGMQ

SEQ ID NO: 35 - protein, 17 aa, Artificial Sequence
  Anti-TROP2 Antibody 2 CDRH2
WINTHSGVPKYAEDFKG

SEQ ID NO: 36 - protein, 12 aa, Artificial Sequence
  Anti-TROP2 Antibody 2 CDRH3
SGFGSSYWYFDV

SEQ ID NO: 37 - protein, 11 aa, Artificial Sequence
  Anti-EGFR Antibody 1 CDRL1
QASQDISNYLN

SEQ ID NO: 38 - protein, 7 aa, Artificial Sequence
  Anti-EGFR Antibody 1 CDRL2
DASNLET

SEQ ID NO: 39 - protein, 9 aa, Artificial Sequence
  Anti-EGFR Antibody 1 CDRL3
QHFDHLPLA

SEQ ID NO: 40 - protein, 7 aa, Artificial Sequence
  Anti-EGFR Antibody 1 CDRH1
SGDYYWT

SEQ ID NO: 41 - protein, 17 aa, Artificial Sequence
  Anti-EGFR Antibody 1 CDRH2
GHIYYSGNTNYNPSLKS

SEQ ID NO: 42 - protein, 9 aa, Artificial Sequence
  Anti-EGFR Antibody 1 CDRH3
DRVTGAFDI

SEQ ID NO: 43 - protein, 11 aa, Artificial Sequence
  Anti-EGFR Antibody 2 CDRL1
HSSQDINSNIG

SEQ ID NO: 44 - protein, 7 aa, Artificial Sequence
  Anti-EGFR Antibody 2 CDRL2
HGTNLDD

SEQ ID NO: 45 - protein, 9 aa, Artificial Sequence
  Anti-EGFR Antibody 2 CDRL3
VQYAQFPWT

SEQ ID NO: 46 - protein, 11 aa, Artificial Sequence
  Anti-EGFR Antibody 2 CDRH1
GYSITSDFAWN

SEQ ID NO: 47 - protein, 16 aa, Artificial Sequence
  Anti-EGFR Antibody 2 CDRH2
GYISYSGNTRYNPSLK

SEQ ID NO: 48 - protein, 9 aa, Artificial Sequence
  Anti-EGFR Antibody 2 CDRH3
VTAGRGFPY

SEQ ID NO: 49 - protein, 214 aa, Artificial Sequence
  Trastuzumab Light Chain
DIQMTQSPSSLSASVGDRVTITCRASQDVNTAVAWYQQKPGKAPKLLIYSASFLYSGVPSRFSGSRSGTDFTLTISSLQPEDFATYYCQQHYTTPPTFGQGTKVEIKRTVAAPSVFIFPPSDEQLKSGTASVVCLLNNFYPREAKVQWKVDNALQSGNSQESVTEQDSKDSTYSLSSTLTLSKADYEKHKVYACEVTHQGLSSPVTKSFNRGEC

SEQ ID NO: 50 - protein, 450 aa, Artificial Sequence
  Trastuzumab Heavy Chain
EVQLVESGGGLVQPGGSLRLSCAASGFNIKDTYIHWVRQAPGKGLEWVARIYPTNGYTRYADSVKGRFTISADTSKNTAYLQMNSLRAEDTAVYYCSRWGGDGFYAMDYWGQGTLVTVSSASTKGPSVFPLAPSSKSTSGGTAALGCLVKDYFPEPVTVSWNSGALTSGVHTFPAVLQSSGLYSLSSVVTVPSSSLGTQTYICNVNHKPSNTKVDKKVEPKSCDKTHTCPPCPAPELLGGPSVFLFPPKPKDTLMISRTPEVTCVVVDVSHEDPEVKFNWYVDGVEVHNAKTKPREEQYNSTYRVVSVLTVLHQDWLNGKEYKCKVSNKALPAPIEKTISKAKGQPREPQVYTLPPSREEMTKNQVSLTCLVKGFYPSDIAVEWESNGQPENNYKTTPPVLDSDGSFFLYSKLTVDKSRWQQGNVFSCSVMHEALHNHYTQKSLSLSPGK

SEQ ID NO: 51 - protein, 450 aa, Artificial Sequence
  Modified HER2 antibody Heavy Chain
EVQLVESGGGLVQPGGSLRLSCAASGFNIKDTYIHWVRQAPGKGLEWVARIYPTNGYTRYADSVKGRFTISADTSKNTAYLQMNSLRAEDTAVYYCSRWGGDGFYAMDYWGQGTLVTVSSASTKGPSVFPLAPSSKSTSGGTAALGCLVKDYFPEPVTVSWNSGALTSGVHTFPAVLQSSGLYSLSSVVTVPSSSLGTQTYICNVNHKPSNTKVDKKVEPKSCDKTHTCPPCPAPEAAGGPSVFLFPPKPKDTLMISRTPEVTCVVVDVSHEDPEVKFNWYVDGVEVHNAKTKPREEQYNSTYRVVSVLTVLHQDWLNGKEYKCKVSNKALPAPIEKTISKAKGQPREPQVYTLPPSREEMTKNQVSLTCLVKGFYPSDIAVEWESNGQPENNYKTTPPVLDSDGSFFLYSKLTVDKSRWQQGNVFSCSVMHEALHNHYTQKSLSLSPGK

SEQ ID NO: 52 - protein, 214 aa, Artificial Sequence
  Pertuzumab Light Chain
DIQMTQSPSSLSASVGDRVTITCKASQDVSIGVAWYQQKPGKAPKLLIYSASYRYTGVPSRFSGSGSGTDFTLTISSLQPEDFATYYCQQYYIYPYTFGQGTKVEIKRTVAAPSVFIFPPSDEQLKSGTASVVCLLNNFYPREAKVQWKVDNALQSGNSQESVTEQDSKDSTYSLSSTLTLSKADYEKHKVYACEVTHQGLSSPVTKSFNRGEC

SEQ ID NO: 53 - protein, 449 aa, Artificial Sequence
  Pertuzumab Heavy Chain
EVQLVESGGGLVQPGGSLRLSCAASGFTFTDYTMDWVRQAPGKGLEWVADVNPNSGGSIYNQRFKGRFTLSVDRSKNTLYLQMNSLRAEDTAVYYCARNLGPSFYFDYWGQGTLVTVSSASTKGPSVFPLAPSSKSTSGGTAALGCLVKDYFPEPVTVSWNSGALTSGVHTFPAVLQSSGLYSLSSVVTVPSSSLGTQTYICNVNHKPSNTKVDKKVEPKSCDKTHTCPPCPAPELLGGPSVFLFPPKPKDTLMISRTPEVTCVVVDVSHEDPEVKFNWYVDGVEVHNAKTKPREEQYNSTYRVVSVLTVLHQDWLNGKEYKCKVSNKALPAPIEKTISKAKGQPREPQVYTLPPSREEMTKNQVSLTCLVKGFYPSDIAVEWESNGQPENNYKTTPPVLDSDGSFFLYSKLTVDKSRWQQGNVFSCSVMHEALHNHYTQKSLSLSPGK

SEQ ID NO: 54 - protein, 449 aa, Artificial Sequence
  Modified HER2 Antibody 2 Heavy Chain
EVQLVESGGGLVQPGGSLRLSCAASGFTFTDYTMDWVRQAPGKGLEWVADVNPNSGGSIYNQRFKGRFTLSVDRSKNTLYLQMNSLRAEDTAVYYCARNLGPSFYFDYWGQGTLVTVSSASTKGPSVFPLAPSSKSTSGGTAALGCLVKDYFPEPVTVSWNSGALTSGVHTFPAVLQSSGLYSLSSVVTVPSSSLGTQTYICNVNHKPSNTKVDKRVEPKSCDKTHTCPPCPAPEAAGGPSVFLFPPKPKDTLMISRTPEVTCVVVDVSHEDPEVKFNWYVDGVEVHNAKTKPREEQYNSTYRVVSVLTVLHQDWLNGKEYKCKVSNKALPAPIEKTISKAKGQPREPQVYTLPPSREEMTKNQVSLTCLVKGFYPSDIAVEWESNGQPENNYKTTPPVLDSDGSFFLYSKLTVDKSRWQQGNVFSCSVMHEALHNHYTQKSLSLSPGK

SEQ ID NO: 55 - protein, 213 aa, Artificial Sequence
  Anti-CDH6 Antibody Light Chain
DIQMTQSPSSLSASVGDRVTITCKASQNIYKNLAWYQQKPGKAPKLLIYDANTLQTGVPSRFSGSGSGSDFTLTISSLQPEDFATYFCQQYYSGWAFGQGTKVEIKRTVAAPSVFIFPPSDEQLKSGTASVVCLLNNFYPREAKVQWKVDNALQSGNSQESVTEQDSKDSTYSLSSTLTLSKADYEKHKVYACEVTHQGLSSPVTKSFNRGEC

SEQ ID NO: 56 - protein, 452 aa, Artificial Sequence
  Anti-CDH6 Antibody Heavy Chain
EVQLVQSGAEVKKPGASVKVSCKASGYTFTRNFMHWVRQAPGQGLEWMGWIYPGDGETEYAQKFQGRVTITADTSTSTAYMELSSLRSEDTAVYYCARGVYGGFAGGYFDFWGQGTLVTVSSASTKGPSVFPLAPSSKSTSGGTAALGCLVKDYFPEPVTVSWNSGALTSGVHTFPAVLQSSGLYSLSSVVTVPSSSLGTQTYICNVNHKPSNTKVDKRVEPKSCDKTHTCPPCPAPEAAGGPSVFLFPPKPKDTLMISRTPEVTCVVVDVSHEDPEVKFNWYVDGVEVHNAKTKPREEQYNSTYRVVSVLTVLHQDWLNGKEYKCKVSNKALGAPIEKTISKAKGQPREPQVYTLPPSREEMTKNQVSLTCLVKGFYPSDIAVEWESNGQPENNYKTTPPVLDSDGSFFLYSKLTVDKSRWQQGNVFSCSVMHEALHNHYTQKSLSLSPGK

SEQ ID NO: 57 - protein, 6 aa, Artificial Sequence
  Pertuzumab CDRL1
QDVSIG

SEQ ID NO: 58 - protein, 3 aa, Artificial Sequence
  Pertuzumab CDRL2
SAS

SEQ ID NO: 59 - protein, 9 aa, Artificial Sequence
  Pertuzumab CDRL3
QQYYIYPYT

SEQ ID NO: 60 - protein, 8 aa, Artificial Sequence
  Pertuzumab CDRH1
GFTFTDYT

SEQ ID NO: 61 - protein, 8 aa, Artificial Sequence
  Pertuzumab CDRH2
VNPNSGGS

SEQ ID NO: 62 - protein, 12 aa, Artificial Sequence
  Pertuzumab CDRH3
ARNLGPSFYFDY

SEQ ID NO: 63 - protein, 11 aa, Artificial Sequence
  Anti-CDH6 Antibody CDRL1
KASQNIYKNLA

SEQ ID NO: 64 - protein, 7 aa, Artificial Sequence
  Anti-CDH6 Antibody CDRL2
DANTLQT

SEQ ID NO: 65 - protein, 8 aa, Artificial Sequence
  Anti-CDH6 Antibody CDRL3
QQYYSGWA

SEQ ID NO: 66 - protein, 5 aa, Artificial Sequence
  Anti-CDH6 Antibody CDRH1
RNFMH

SEQ ID NO: 67 - protein, 17 aa, Artificial Sequence
  Anti-CDH6 Antibody CDRH2
WIYPGDGETEYAQKFQG

SEQ ID NO: 68 - protein, 13 aa, Artificial Sequence
  Anti-CDH6 Antibody CDRH3
GVYGGFAGGYFDF